European Patent Application EP 4 169 931 A1, published April 26, 2023. Title: NUCLEIC ACID LIGAND AND USE THEREOF. Applicant: NUHIGH BIOTECHNOLOGIES CO.,LTD. Application EP21828968.4. The sequence listing filed with the application follows.

SEQUENCE LISTING (28 sequences)

SEQ ID NO: 1 - DNA, 31 bp, Artificial Sequence
tcgaacggtatatatattaatatatatatac

SEQ ID NO: 2 - DNA, 15 bp, Artificial Sequence
tcgaacgggtatacc

SEQ ID NO: 3 - DNA, 17 bp, Artificial Sequence
tcgaacgggatatatcc

SEQ ID NO: 4 - DNA, 19 bp, Artificial Sequence
tcgaacgggattataatcc

SEQ ID NO: 5 - DNA, 21 bp, Artificial Sequence
tcgaacgggatatatatatcc

SEQ ID NO: 6 - DNA, 27 bp, Artificial Sequence
tcgaacgggatatactatagtatatcc

SEQ ID NO: 7 - DNA, 29 bp, Artificial Sequence
tcgaagtgtatatactatagtatatacac

SEQ ID NO: 8 - DNA, 31 bp, Artificial Sequence
tcggagtgtatatactatagtatatacactc

SEQ ID NO: 9 - DNA, 32 bp, Artificial Sequence
tcggagtgtatatactatagtatatacactcc

SEQ ID NO: 10 - DNA, 33 bp, Artificial Sequence
tgagagtgtatatactatagtatatacactctc

SEQ ID NO: 11 - DNA, 34 bp, Artificial Sequence
ggagagtgtatatactatagtatatacactctcc

SEQ ID NO: 12 - DNA, 38 bp, Artificial Sequence
gaggagttcagtagcatgagctgtgtagacgtatatac

SEQ ID NO: 13 - DNA, 10 bp, Artificial Sequence
tatatacgtc

SEQ ID NO: 14 - DNA, 13 bp, Artificial Sequence
tatatacgtctac

SEQ ID NO: 15 - DNA, 15 bp, Artificial Sequence
tatatacgtctacac

SEQ ID NO: 16 - DNA, 18 bp, Artificial Sequence
tatatacgtctacacagc

SEQ ID NO: 17 - DNA, 20 bp, Artificial Sequence
tatatacgtctacacagctc

SEQ ID NO: 18 - DNA, 24 bp, Artificial Sequence
tatatacgtctacacagctcatgc

SEQ ID NO: 19 - DNA, 27 bp, Artificial Sequence
tatatacgtctacacagctcatgctac

SEQ ID NO: 20 - DNA, 32 bp, Artificial Sequence
tatatacgtctacacagctcatgctactgaac

SEQ ID NO: 21 - DNA, 27 bp, Artificial Sequence
tcgaacgggacggctggctgtgtgtgt

SEQ ID NO: 22 - DNA, 10 bp, Artificial Sequence
ccagccgtcc

SEQ ID NO: 23 - DNA, 27 bp, Artificial Sequence
ttgatgactgatcatgcatgatcagtc

SEQ ID NO: 24 - DNA, 31 bp, Artificial Sequence; identical to SEQ ID NO: 1

SEQ ID NO: 25 - DNA, 23 bp, Artificial Sequence
tcgaacggattacagctgtaatc

SEQ ID NO: 26 - DNA, 21 bp, Artificial Sequence
tcgaacggctacagctgtagc

SEQ ID NO: 27 - DNA, 17 bp, Artificial Sequence
tcgaacgggatatatcc

SEQ ID NO: 28 - DNA, 15 bp, Artificial Sequence
tcgaacgggtatacc